European Patent Application EP 4 400 519 A1, published July 17, 2024. Title: BISPECIFIC NK CELL AGONIST, PREPARATION METHOD, AND APPLICATION. Applicant: SHANGHAI NK CELL TECH CO., LTD. The sequence listing filed with the application follows.

SEQUENCE LISTING (10 sequences)

SEQ ID NO: 1 - protein, 120 aa, Artificial Sequence
  amino acid sequence of VH region of CD16A single chain antibody
QVQLVQSGAEVKKPGESLKVSCKASGYTFTSYYMHWVRQAPGQGLEWMGIINPSGGSTSYAQKFQGRVTMTRDTSTSTVYMELSSLRSEDTAVYYCARGSAYYYDFADYWGQGTLVTVSS

SEQ ID NO: 2 - protein, 106 aa, Artificial Sequence
  amino acid sequence of VL region of CD16A single chain antibody
SYVLTQPSSVSVAPGQTATISCGGHNIGSKNVHWYQQRPGQSPVLVIYQDNKRPSGIPERFSGSNSGNTATLTISGTQAMDEADYYCQVWDNYSVLFGGGTKLTVL

SEQ ID NO: 3 - protein, 15 aa, Artificial Sequence
  amino acid sequence of the first linker
GGGGSGGGGSGGGGS

SEQ ID NO: 4 - protein, 14 aa, Artificial Sequence
  amino acid sequence of the second linker
GGGGSGGGGSGGGG

SEQ ID NO: 5 - protein, 184 aa, Artificial Sequence
  amino acid sequence of 4-1BBL extracellular domain
REGPELSPDDPAGLLDLRQGMFAQLVAQNVLLIDGPLSWYSDPGLAGVSLTGGLSYKEDTKELVVAKAGVYYVFFQLELRRVVAGEGSGSVSLALHLQPLRSAAGAAALALTVDLPPASSEARNSAFGFQGRLLHLSAGQRLGVHLHTEARARHAWQLTQGATVLGLFRVTPEIPAGLPSPRSE

SEQ ID NO: 6 - protein, 20 aa, Artificial Sequence
  amino acid sequence of the third linker
GGGGSGGGGSGGGGSGGGGS

SEQ ID NO: 7 - protein, 20 aa, Artificial Sequence
  amino acid sequence of the fourth linker
GGGGSGGGGSGGGGSGGGGS

SEQ ID NO: 8 - protein, 853 aa, Artificial Sequence
  amino acid sequence of fusion protein
QVQLVQSGAEVKKPGESLKVSCKASGYTFTSYYMHWVRQAPGQGLEWMGIINPSGGSTSYAQKFQGRVTMTRDTSTSTVYMELSSLRSEDTAVYYCARGSAYYYDFADYWGQGTLVTVSSGGGGSGGGGSGGGGSSYVLTQPSSVSVAPGQTATISCGGHNIGSKNVHWYQQRPGQSPVLVIYQDNKRPSGIPERFSGSNSGNTATLTISGTQAMDEADYYCQVWDNYSVLFGGGTKLTVLGGGGSGGGGSGGGGREGPELSPDDPAGLLDLRQGMFAQLVAQNVLLIDGPLSWYSDPGLAGVSLTGGLSYKEDTKELVVAKAGVYYVFFQLELRRVVAGEGSGSVSLALHLQPLRSAAGAAALALTVDLPPASSEARNSAFGFQGRLLHLSAGQRLGVHLHTEARARHAWQLTQGATVLGLFRVTPEIPAGLPSPRSEGGGGSGGGGSGGGGSGGGGSREGPELSPDDPAGLLDLRQGMFAQLVAQNVLLIDGPLSWYSDPGLAGVSLTGGLSYKEDTKELVVAKAGVYYVFFQLELRRVVAGEGSGSVSLALHLQPLRSAAGAAALALTVDLPPASSEARNSAFGFQGRLLHLSAGQRLGVHLHTEARARHAWQLTQGATVLGLFRVTPEIPAGLPSPRSEGGGGSGGGGSGGGGSGGGGSREGPELSPDDPAGLLDLRQGMFAQLVAQNVLLIDGPLSWYSDPGLAGVSLTGGLSYKEDTKELVVAKAGVYYVFFQLELRRVVAGEGSGSVSLALHLQPLRSAAGAAALALTVDLPPASSEARNSAFGFQGRLLHLSAGQRLGVHLHTEARARHAWQLTQGATVLGLFRVTPEIPAGLPSPRSEHHHHHH

SEQ ID NO: 9 - DNA, 2559 bp, Artificial Sequence
  nucleotide sequence encoding the fusion protein without codon optimization
caagttcaattggttcaatctggtgctgaggttaagaaaccaggtgagtctttgaaggtttcttgtaaggcttctggttatactttcacttcttactatatgcattgggttagacaagctccaggtcaaggtttggagtggatgggtattattaatccatctggtggttctacttcttatgctcaaaagttccaaggtagagttactatgactagagatacttctacttctactgtttatatggagttgtcttctttgagatctgaagatactgctgtttattattgtgctagaggttctgcttattattatgatttcgctgattattggggtcaaggtactttggttactgtctcttctggtggtggtggttctggtggtggtggttctggtggtggtggttcctcttacgtcttgactcaaccatcttctgtctctgttgctccaggtcaaactgctactatttcttgtggtggtcataatattggttctaagaatgttcattggtatcaacaaagaccaggtcaatctccagtcttggtcatctatcaagataacaagagaccatctggtattccagagagattctctggttctaattctggtaatactgctactttgactatttctggtactcaagctatggatgaagctgattactattgtcaagtttgggataattattctgtcttgttcggtggtggtactaagttgactgttttgggtggtggtggttctggaggtggcggttctggtggtggtggtcgcgagggtcccgagctttcgcccgacgatcccgccggcctcttggacctgcggcagggcatgtttgcgcagctggtggcccaaaatgttctgctgatcgatgggcccctgagctggtacagtgacccaggcctggcaggcgtgtccctgacggggggcctgagctacaaagaggacacgaaggagctggtggtggccaaggctggagtctactatgtcttctttcaactagagctgcggcgcgtggtggccggcgagggctcaggctccgtttcacttgcgctgcacctgcagccactgcgctctgctgctggggccgccgccctggctttgaccgtggacctgccacccgcctcctccgaggctcggaactcggccttcggtttccagggccgcttgctgcacctgagtgccggccagcgcctgggcgtccatcttcacactgaggccagggcacgccatgcctggcagcttacccagggcgccacagtcttgggactcttccgggtgacccccgaaatcccagccggactcccttcaccgaggtcggaaggtggtggtggttctggaggtggcggttctggtggtggtggttctggaggtggcggttctcgcgagggtcccgagctttcgcccgacgatcccgccggcctcttggacctgcggcagggcatgtttgcgcagctggtggcccaaaatgttctgctgatcgatgggcccctgagctggtacagtgacccaggcctggcaggcgtgtccctgacggggggcctgagctacaaagaggacacgaaggagctggtggtggccaaggctggagtctactatgtcttctttcaactagagctgcggcgcgtggtggccggcgagggctcaggctccgtttcacttgcgctgcacctgcagccactgcgctctgctgctggggccgccgccctggctttgaccgtggacctgccacccgcctcctccgaggctcggaactcggccttcggtttccagggccgcttgctgcacctgagtgccggccagcgcctgggcgtccatcttcacactgaggccagggcacgccatgcctggcagcttacccagggcgccacagtcttgggactcttccgggtgacccccgaaatcccagccggactcccttcaccgaggtcggaaggtggtggtggttctggaggtggcggttctggtggtggtggttctggaggtggcggttctcgcgagggtcccgagctttcgcccgacgatcccgccggcctcttggacctgcggcagggcatgtttgcgcagctggtggcccaaaatgttctgctgatcgatgggcccctgagctggtacagtgacccaggcctggcaggcgtgtccctgacggggggcctgagctacaaagaggacacgaaggagctggtggtggccaaggctggagtctactatgtcttctttcaactagagctgcggcgcgtggtggccggcgagggctcaggctccgtttcacttgcgctgcacctgcagccactgcgctctgctgctggggccgccgccctggctttgaccgtggacctgccacccgcctcctccgaggctcggaactcggccttcggtttccagggccgcttgctgcacctgagtgccggccagcgcctgggcgtccatcttcacactgaggccagggcacgccatgcctggcagcttacccagggcgccacagtcttgggactcttccgggtgacccccgaaatcccagccggactcccttcaccgaggtcggaacatcatcaccatcaccat

SEQ ID NO: 10 - DNA, 2559 bp, Artificial Sequence
  codon-optimized nucleotide sequence encoding the fusion protein
caagttcagttggtgcaatctggtgctgaggttaagaaaccaggtgagtcattgaaggtttcctgtaaagcctctggttatactttcacctcatactatatgcattgggttcgacaagctccaggtcaaggtttagagtggatgggtataattaatccctctggtggaagcacttcctatgctcagaagttccaaggtcgggtaactatgacccgtgatacaagcacatctacagtgtatatggagctgtcgagtttaaggagtgaggacactgctgtttattactgtgcgcgcggttcagcatactattacgatttcgccgactactggggtcaaggaactttagtaacagtctcttctggaggtggaggttctggtggaggtggatctggtggaggtggatcctcttacgtcttgactcaaccctcttctgtctccgtagctccaggtcaaactgccacaattagctgtggcgggcataatataggtagtaagaatgttcattggtatcaacagcggccaggtcagtcacccgttctcgtcatctaccaggataacaagcgccccagtggtattcctgagcgtttctctggtagcaattcgggtaatactgctacgttgacaattagcggtactcaagctatggacgaggcggattactattgccaagtttgggataattattccgtcctcttcggtgggggtactaagcttacagtgttaggtggaggtggatctggaggtggcggttctggtggaggtggaagagagggaccagaattgtccccagatgaccctgctggcttattggaccttagacaaggaatgtttgcccagttagtagctcaaaacgttctacttatcgatggtccactttcatggtattcagatccagggttggcgggcgtcagcctgaccggtggactgagttacaaagaagatactaaggagttggttgtagctaaagcaggagtttactatgtgtttttccaactcgaactaagacgagttgtggccggtgaagggtcggggtctgtctccttggctctacacttacaaccccttcgttcagctgccggagcagcagccctggctctgacagttgacttgccacctgcatcctcagaagcacgtaacagtgcttttggatttcaaggcagattgctacatttatccgcagggcagagactcggagtgcacttgcacacggaggctagagccaggcatgcttggcagttgacccagggcgctactgtcttgggtctgttcagagttacccctgaaattcctgccggacttccttcgccgaggagtgaaggtggaggtggttctggtggaggtggatctggtggaggtggatctggtggtggaggttctagagagggaccagaattgtccccagatgaccctgctggcttattggaccttagacaaggaatgtttgcccagttagtagctcaaaacgttctacttatcgatggtccactttcatggtattcagatccagggttggcgggcgtcagcctgaccggtggactgagttacaaagaagatactaaggagttggttgtagctaaagcaggagtttactatgtgtttttccaactcgaactaagacgagttgtggccggtgaagggtcggggtctgtctccttggctctacacttacaaccccttcgttcagctgccggagcagcagccctggctctgacagttgacttgccacctgcatcctcagaagcacgtaacagtgcttttggatttcaaggcagattgctacatttatccgcagggcagagactcggagtgcacttgcacacggaggctagagccaggcatgcttggcagttgacccagggcgctactgtcttgggtctgttcagagttacccctgaaattcctgccggacttccttcgccgaggagtgaaggtggaggtggatctggtggaggtggctctggtggcggtggttctggtggcggtggctctagagagggaccagaattgtccccagatgaccctgctggcttattggaccttagacaaggaatgtttgcccagttagtagctcaaaacgttctacttatcgatggtccactttcatggtattcagatccagggttggcgggcgtcagcctgaccggtggactgagttacaaagaagatactaaggagttggttgtagctaaagcaggagtttactatgtgtttttccaactcgaactaagacgagttgtggccggtgaagggtcggggtctgtctccttggctctacacttacaaccccttcgttcagctgccggagcagcagccctggctctgacagttgacttgccacctgcatcctcagaagcacgtaacagtgcttttggatttcaaggcagattgctacatttatccgcagggcagagactcggagtgcacttgcacacggaggctagagccaggcatgcttggcagttgacccagggcgctactgtcttgggtctgttcagagttacccctgaaattcctgccggacttccttcgccgaggagtgaacatcatcatcaccatcat